European Patent Specification EP 3 679 158 B1, published April 30, 2025. Title: Single Immunoglobulin Interleukin-1 Receptor Related (SIGIRR) Variants And Uses Thereof. Applicant: Regeneron Pharmaceuticals, Inc. The sequence listing filed with the application follows.

SEQUENCE LISTING (16 sequences)

SEQ ID NO: 1 - DNA, 11739 bp, Homo sapien
  genomic wild type SIGIRR
actgcggggcggggccgcacctgctgccgctgccggggctacgccgccgccggggctgttgccgctgcgcacctggctcaggtgagctgccccgcccccgcccggcgcgagccccaggtcctggcagcaggtgagtggcggtcgccatcagacccgcgaaggtgagtggaggtcgcagtcctcccagagccgctgcaggcctggagtcggggcccggggcgctgcttgtccctgggcgcggtctctcaggaaatggctcggggccggggaggttcccgcgtcgcccggaagcccgagctcgcccgcgtcctggccctttccagggctgggggaagggaggaaagtgggcgaagggggcgggggccaccctttcctctgcccgacgtggtcagcggctttttggtgaccctcgcgcagaacagagcggggctaggagcgccgaggcgcgcagggatcccacctcggtcgcccaagcctggatcccagctcgaggcttcctgaggcgccgagggcggaccaagagtcaggctggggcccgagctcgcccggcgccgggtggagcttccgccatccgcgcgcctctgccccggccgagcgccccgagccgcacccccgtgcccgcctcccgcgcgcgtcctcgttctccgccctcctcacttggagggcgcccagggcgcaggtgggcgcggggtaggggagcgaaccagagcccctcggcctgcggggccgcagccttttacccacgttcctgcttcaggacaggcgctgggggcccagcgcgcacggggagcggaggggcggcgcgtccgagctgagcgggagtcgcccgcagggtgctgggtgctgagcgtcgaacccaccgggcaggggcggccgcggaccgaggacgctggctgggtctgagggcgggaggagctggcgctttctaagaacctcaaggtgcccagcagagtgcggtgggcagtgcgaggcgaccagggccaggcttggactgagattctgggcgcctcggaagagctgtgcgggcgagggtcggagactttgtgggtgttcatgctcaccctggacggtggacctgggggctcgggggtgcaggacgttagcagagagagggaaggagagggtgccaagccagccctgagagatggtgacgctgagaccgggtgcacagagcagccgccgagccggggcttcacagttggcggctgaccccagggcctgtgctggaggccctgctcctgcttcctgcgggggtgccctgggccctgctgtgcctgcttcctgacctgcagtgtggggagaaccttcttgaggggcttccaaggacccacttcaaggaggggctggtaccaggctctgtgggggaaggggtgctgtctttgggaccctgagcccaaggcccaccatcacccaaggctgagtaccgggacaaaggaaggtcctagcagggctgggactcagtcagacaagtacctgtagaaagcctgctgctgagagggtgctcagccagggccgggaggctggatggcagccctccacaatgaagccctgcccccatgtggctgagggcagggccagggtccaaaggagacccttgtctgattctgtgggcaataccagccaccggtcactgggtccccagtcccaggtcaacctggggagtgtcagtttggtgacaacaggagatgccatctgcccctcatctgctctgagccaggagcctcggccacctgtgtttgctccttatttggaaaagggggcgctgccctcccaccccagcctgaagggaaggtccacaagatgccatagtcccttgtaactgctcacccatcgggggagctatgtctgggagagggacggggagagggcggaagagttctgctggagccccattgttgaccgggagtttctgaaggccctgttccccggggtcagaggtcaaagacacatgggggagcaaaccggccccttggctcctgagtgtgagctctagtagcgtctggaaggcatgccgcgcggtccccggtcctccttgtatgtgtgcagggtggccctggcgggggtctcctggctggaggaccccccatgcattacccctggaacctgcccctttgagcaccccccaccccacaacacacacgcacacacacaaacgcacgcacacgcacatactgcacacacattgcacacacgcagacacactgcacacacacacacacacacacacacacacacacacacacacacgctgcacagaggaaagtgccgtgcctgggtgggttggggcgggctccagaggaaggagccgcttgactcagagctacaggaagagccggggcaggcggggtgagaaccaccaactgcccgtcctcccgcccgcctagggaaggggtgggtgcctgggtggggtttagggttaggagaggatgtgactgcaaggccaggaagctacagggaaagttctgatcaaaatacacaaagacacaagccaggtccccaccgcgcttggcgatgcatccatagcagccttggtgctgtggacactccctggggcccagcgaaggggagagtttgctcccaaaggcgcaccaatgaccaacatttgccccccggaggaaagaactggaaccaggtgactgccttccccgctgctctgagtgagcctgtgtcagggcctggctgagaggaggcccacggcgcccaagacccatatgcatgtgtgtgcatgtgtgtgtgagacagagcgaggggcagcaggaggctgtgtcgcatcagcggccaagggtgggtgtcaggtgcagtgtgtgtgctgtggggtgcctgtggtcctaggctctgtgacaagcgttgcaatgggtgttgtatatactcaacagttgtgtgaggggtctgcagcctaagctgtgtgcagtggtaatgggaggtgtgtgtggtaggaagtgtgctgtgtaggaggtgcaagtgtgcacacgggctgagactgaagctctgtgcaggtgcacatgggccagagggctgtgtgtatgtgatgtgtgcaggggaggaggggcagaggagagggtgcaggggaagttagggaggggagggggtacaaggaaaggtgtgcaggggagagggtgcagggaaaggtggggaggggagagggtgcaggggaaggtaggcagaggagagggtgcaggggagagggtgcaggggaaggtgtgcagggaaaggtggggaggggagagggtgcaggggaaggtaggcagaggagagggtgcaggggaaggtgtgcaggggagagggtgcagggaaaggtggggaggggagagggtgcaggggaaggtaggcagaggagagggtgcaggggaaggtgtgcagggaaaggtggggagggagagggtgcaggggaaggtaggcagaggagagagtgcaggggaaggtgtgcaggggagagggtgcagggaaaggtggggaggggagagggtgcaggggaaggtaggcagacgagagtacagggaaaggtagggaggagagaaggtgcaggaggaggcaggcagaagagagggtgcaggggaaggtggggaggggagagggtgcagggggaggcaggcagaggagagggttcaggggagagggtgcaggggaaggtgggcaggggaaggtggggagtggagagcgtgcagggggaggcaggcagaggagagggtgcaggggaaggtgcgtaggggagagggagcaggggagagggtgcgggaagagggtgcaggggagggtttgcagggagagggtgcaggggagagggtgcaaggagaggcaggcagcggagagggtgcagaggagggtttgcaggggagggcacctgctttcttgctgtgctcgtatcctggcagtctgcccttgacttccagaaggctctgaggctgcttttggagggaggactttgaggtctgagcttggggcggtcacggaagcactgcaggagatgccaggggttctgctgggctggcggtgtgacctcccgggcttgctgtgaggggttggtttcctgggaagtgtgtgctttaaggaccctcagtgggtggttcccctgggtcaaggactttccttggagtgtcctccaccgcaaaggacttcttcaaggaccccctggccatcccccatgggtgtgtgcctcatgctgtatcggttcccgaggaaactgccaaacagtcaaacctggggcctctggctgtgcttcacccatggagagggaataggtggcaggctaagaggactgtccctgccactgcctctggggccttagcggggaggaatcctgagggagctggggtgcagaaacttaggcttgatccccacatccccacttccactgtgtccctgcagcagggaggggagtagacagtcagtgcctgttggataaacagggtgaccctgtggcatccagtgaggagaggcccctggggccctgggctgccaaggaagaggctctgggcttctccctgcagccacctcactgaggagctttgggagacttgaggtgtgtgtggctgctgctacgggctgggaaaggacatgggacccgagacctccatccccaccgggcgctgttcaccctccggcctcacaaccgcagggcgaggctaagctgagggttcccgaggtgtttcccgaggtgtttcgaggtgtctgtgctcacgtgcactcctgactgtaaccagacgtgggccagagctgggcaccccccctcgactgcatccagacatggttagagctgggcaccccccccccccgactgtatccagacatggtcagagctgagcacccctccccgactgtatccagacatgttcagagctgggcacccccccccgactgtatccagacatgttcagagctgggcacccccccccgactgtatccagacatggtcagagctgggcacccccccccgactgtatccagacatggtcagagctgggcaccccccgactgcatccagacatggtcagagctgagcacccccccccgcccgactgtatccagacatggtcagagctgggcaccccccgactgcatccagacatggtcagagctgggcacccccctccccgactgcattcagacatggtcagagctgggcacccccgccgactgcatccagacatggtcagagttgggcaccccccccccgactgtatccagacatggtcagagctgggcaccccccgactgcatccagacatggtcagagctgggcacccctccccgactgtatccagacatggtcagagctgggcacccccccccgactgtatccagacatggtcagagctgggcacctccccccgactgtatccagacatggtcagagctgggcacctcccccgactgcatccagacatggtcagagctgggcaccccccccgactgcatccagacatggtcagagctgggcaccccccccccccactgtatccagacatggtcagagctgggcacccccctccccgactgcatccagacatggtcagagctgagcaccccccccccccgactgtatccagacatggtcagagctgggcacccccctccccgactgtatccagacatggtcagagctgagccccccccccgcccgactgtatccagacatggtcagagctgggcaccccccgactgcatccagacatggtcagagctgagcacccctccccgactgcatccagacatggtcagagctgggcaccccccccccccaccgactgtatccagacatggtcagagctgggcaacccccaccgactgtatccagacatggtcagagctgggcaccccccgactgcatccagacatggtcagagctgggcaccccccgccgactgtatccagacatggtcagagctgggcacccccctccccgactgcatccagacatggtcagagctgggcacccccctccccgactgcatccagacatggtcagagctgggcacccctccccgactgtatccagacatggtcagagctgggcacccccctccccgactgtatccagacatggtcagagctgggcacccccgccgactgtatccagacatggtcagagctgggcaccccccgactgcatccagacatggtcagagctgggcacccctccccgactgtatccagacatggtcagagctgggcaccccccccccccgactgtatccagacatggtcagagctgagcacccctccccgactgtatccagacatgttcagagctgggcacccccccccccgactgtatccagacatggtcagagctgggcacccccctccccgactgcatccagacatggtcagagctgagcaccccccccgcccgactgcatccagacatggtcagagctgggcaccccccgactgcatccagacatggtcagagctgggcacccccctccccgactgcattcagacatggtcagagctgggcacccccctccccgactgcatccagacatggtcagagctgggcacccccgccgactgtatccagacatggtcagagctgggcacccccctccccgactgtatccagacatggtcagagctgggcacccccgccgactgtatccagacatggtcagagctgggcacccccctccccgactgcatccagacatgttcagagctgggcacccccccccgactgtatccagacatggtcagagctgggcaccccccgactgcatccagacatggtcagagctgggcaaccccctccctgactgcatccagacatggtcagagctgggcaccccccccggctgtatccagacatggtcagagctgggcaccccccccccccgactgcatccagacatggtcagagctaagcaaagccccccgccgactgtatccagacatggtcagagctgggcacccccaccccaactgcatccagacatggtcagagctgagcaccccccaccgactgtatccagacatggtcagagctgggcatctcccatggtgtaggttacatcactcacacccctgccccaaggccaggctgtgtctctggcactgcagcaccccctgcagtggcagctctgttgaaggggacagccaggagtgaggccaactgccatgtcgggagacagggtcccacctagtgttcgtccactgcaccctggggccgtcatggtggccccagggccggtggaggtgatcctggacttgatggcccctccccgtggtcctgggctgcgtgaagtggtgcccattctggccacgtgtgaggggctcaaagagacaccctgctggcctccgagaactctgccagcatccatgcggctgctcagggtcgcatctggtcagggccagtgctgtctgtggccggcagttactggttaactcatcctgttcctgtttaacttgttccctggggatggcggcagcctctgacctgtccaggtgccctgtccagctgactgcaaggacagagaggagtcctgcccagctcttggatcagtctgctggccgaggagcccggtggagccaggggtgaccctggagcccagcctgccccgaggaggccccggctcagagccatgccaggtaggcaggtcagagagggatgggcttgaattccccactcccacctcctgcccctcaggctggctccacattgtgcatcctgctcttatcccaggcactctgcctggccacatgccgggggtacaaaggcccctgctcacccctcccactgggcccttggccctgaaaccagggcgagtggtgaggatgagccctgcaccctctcctgccccagaccaggctcatgagggtcagtaaagcccaggaatgctaggagtgggcactgctggggcccacagcagggtgtggccgatgtgagctggcaggagaccataccctactgagaagatggtggtttgacctcccgctagggctcatcaccctgatgtaaagatgaacaagttcaggcctcaggtggtggggagggcttgcctgtggccaggagcagagggccccaagacccccaaggcaggaatgaggccaactgctccaggctcccagctgtgcccatccaggtggaaggtgctggcacactgggcatctgggtccccaaacccactggtgcccacactctctgcagattccccagcagaggcaggccaggctgaggggtgcagtgcccggcccctcctatgagacaggcatcatggtgtcaccaggggtgggcaacaggtgcatctgggaaatggggggctggactcacatcctgggtggacaagcagccagatggggcttgagcgtgggcctggggcagctcaactgtggccactgctctctgtcccctcagcacagggtgggcggaacacccaaagcctggccactactggggaaagacgtgccaagtgctaagcctgtccccatgggactcgtggacagacatggtgtgactgccaagccacacagaggccttatttcttcctgcaccacggaccactgtggaggtggtggggccaggcaccctggcacagctgacccactgtgtcctctctcttcaggtgtctgtgatagggcccctgacttcctctccccgtctgaagaccaggtgctgaggcctgccttgggcagctcagtggctctgaactgcacggcttgggtagtctctgggccccactgctccctgccttcagtccagtggctgaaagacgggcttccattgggaattgggggccactacagcctccacgagtactcctggtaagagacccgggtatccagggtcagagtgacctctcagacatgccaagggcagtggtctccctgacctatgcctgggtctgtaaccacctggccagacatgtcacgagcagagtgcctctgtggacccagacggagggtcagtaatgtcagggacagacccttgggtctgcatggcccctgtaggcacacacctcgtaactgcccagggctacgggtgtcagcaaagtctagggtctgaatgaacaccgaccagctggccaagtctgtgatcaaaggacctccaggccccagacccaggactgggacggctgttctgaaacaaatctgcatcccctccaggttcaggtcacttctcttggcttaaggcccaagaaccacccaggaggcccaattctgcagcctccctgggtgaacccagacaggtggggttcgggggtgtccactggtatccccagtcgaccctgaccctggcttggtatccccagggtcaaggccaacctgtcagaggtgcttgtgtccagtgtcctgggggtcaacgtgaccagcactgaagtctatggggccttcacctgctccatccagaacatcagcttctcctccttcactcttcagagagctggtgatgggggttccccaaggtggagggtagaaggggacctagacctagtgaggcccagggatcttgaggcttgggggctgctggaggggcagcggctcaggcaacccatccgcaggccctacaagccacgtggctgcggtgctggcctccctcctggtcctgctggccctgctgctggccgccctgctctatgtcaagtgccgtctcaacgtgctgctctggtaccaggacgcgtatggggaggtggagataaacggtgcgtggggcccgcgtgggcgcgaggaggggtcgccacggcctccctgagagtgcgctgctgagctcggctttggaggcgtgcggcggggaggggttagcccccgggtgctctgtgcggcccggctggggttaaagtccggggcgggtctgcccctgtgcacgtgggagatggttaggggtgttggggaccccgagggctggtgtgaggcctcgggagccatcggggtgactggccgccgtccgcagacgggaagctctacgacgcctacgtctcctacagcgactgccccgaggaccgcaagttcgtgaacttcatcctaaagccgcagctggagcggcgtcggggctacaagctcttcctggacgaccgcgacctcctgccgcgcgctggtatcccgggccccaccccgtgccccgcccacccggagggcccgccccgccccgccccatgctccgtcccacccggggccccacccccaccatcgagctccgcccccatccccgcccacccgaggccccgcctcaaaaacccgcccaccccgcaggccccgcccctcccttagagctctgcgtccggcaccgcccctgagcctccggccccgccctcccccgcccccgcccctgcgccgccgacgcccgccctcccgcagagccctccgccgacctcttggtgaacctgagccgctgccgacgcctcatcgtggtgctttcggacgccttcctgagccgggcctggtgcagccacagcttccggtgggtcccgcgcggggttgggtgggccccagcgtagcacccacccccctgacggtcccgccccgcagggagggcctgtgccggctgctggagctcacccgcagacccatcttcatcaccttcgagggccagaggcgcgaccccgcgcacccggcgctccgcctgctgcgccagcaccgccacctggtgaccttgctgctctggaggcccggctccgtggtgcggagcaggcgcgggagggtccggggctagcggcgggttagagatgggcggtgcccgggctccaggctgggacccctccgtggggagctctgcggcaccacgctttgtgaatgggccctggggggaggttccgctgcctggggccccgatgcggggagccgcccttgaggcccccggagccacggaatagctgtcgcagggcgtggaacccgtgggcagccgcaggtgtgctcttgggggccaggacgccaggggcttccgaggtgttcacacctgcaaaccgccccgacctggcccccagactccttcctccgatttttggaaagaagtgcagctggcgctgccgcggaaggtgcagtacaggcctgtggaaggagacccccagacgcagctgcaggacgacaaggaccccatgctgattcttcgaggccgagtccctgagggccgggccctggactcagaggtggacccggaccctgagggcgacctgggtatgcccgcccagccccactccccaactggagaagctcagcacagggcggagtgggggcaggcacagggcacagggcctggaggggctccaggtgttgaggactcttcccggcaccgggagcccctgcacggcctctgccctggaggtgctcggccctcggtctgcctgggaacttcctgggcctcacaggccatcacagcagggggtgagcaggggcagcccctggcagtgggtctgggccaaggctgtgggtggccacctcaggcgtctcggtctccccaccccaggtgtccgggggcctgtctttggagagccatcagctccaccgcacaccagtggggtctcgctgggagagagccggagcagcgaagtggacgtctcggatctcggctcgcgaaactacagtgcccgcacagacttctactgcctggtgtccaaggatgatatgtagctcccaccccagagtgcaggatcatagggacagcgggggccagggcagcggcgtcgctcctctgctcaacaggaccacaacccctgccagcagccctgggaccctgccagcagccctgggaaaaggctgtggcctcagggcgcctcccagtgccagaaaataaagtccttttggattctg

SEQ ID NO: 2 - DNA, 11738 bp, Homo sapien
  Variant SIGIRR genomic (c.557delA)
actgcggggcggggccgcacctgctgccgctgccggggctacgccgccgccggggctgttgccgctgcgcacctggctcaggtgagctgccccgcccccgcccggcgcgagccccaggtcctggcagcaggtgagtggcggtcgccatcagacccgcgaaggtgagtggaggtcgcagtcctcccagagccgctgcaggcctggagtcggggcccggggcgctgcttgtccctgggcgcggtctctcaggaaatggctcggggccggggaggttcccgcgtcgcccggaagcccgagctcgcccgcgtcctggccctttccagggctgggggaagggaggaaagtgggcgaagggggcgggggccaccctttcctctgcccgacgtggtcagcggctttttggtgaccctcgcgcagaacagagcggggctaggagcgccgaggcgcgcagggatcccacctcggtcgcccaagcctggatcccagctcgaggcttcctgaggcgccgagggcggaccaagagtcaggctggggcccgagctcgcccggcgccgggtggagcttccgccatccgcgcgcctctgccccggccgagcgccccgagccgcacccccgtgcccgcctcccgcgcgcgtcctcgttctccgccctcctcacttggagggcgcccagggcgcaggtgggcgcggggtaggggagcgaaccagagcccctcggcctgcggggccgcagccttttacccacgttcctgcttcaggacaggcgctgggggcccagcgcgcacggggagcggaggggcggcgcgtccgagctgagcgggagtcgcccgcagggtgctgggtgctgagcgtcgaacccaccgggcaggggcggccgcggaccgaggacgctggctgggtctgagggcgggaggagctggcgctttctaagaacctcaaggtgcccagcagagtgcggtgggcagtgcgaggcgaccagggccaggcttggactgagattctgggcgcctcggaagagctgtgcgggcgagggtcggagactttgtgggtgttcatgctcaccctggacggtggacctgggggctcgggggtgcaggacgttagcagagagagggaaggagagggtgccaagccagccctgagagatggtgacgctgagaccgggtgcacagagcagccgccgagccggggcttcacagttggcggctgaccccagggcctgtgctggaggccctgctcctgcttcctgcgggggtgccctgggccctgctgtgcctgcttcctgacctgcagtgtggggagaaccttcttgaggggcttccaaggacccacttcaaggaggggctggtaccaggctctgtgggggaaggggtgctgtctttgggaccctgagcccaaggcccaccatcacccaaggctgagtaccgggacaaaggaaggtcctagcagggctgggactcagtcagacaagtacctgtagaaagcctgctgctgagagggtgctcagccagggccgggaggctggatggcagccctccacaatgaagccctgcccccatgtggctgagggcagggccagggtccaaaggagacccttgtctgattctgtgggcaataccagccaccggtcactgggtccccagtcccaggtcaacctggggagtgtcagtttggtgacaacaggagatgccatctgcccctcatctgctctgagccaggagcctcggccacctgtgtttgctccttatttggaaaagggggcgctgccctcccaccccagcctgaagggaaggtccacaagatgccatagtcccttgtaactgctcacccatcgggggagctatgtctgggagagggacggggagagggcggaagagttctgctggagccccattgttgaccgggagtttctgaaggccctgttccccggggtcagaggtcaaagacacatgggggagcaaaccggccccttggctcctgagtgtgagctctagtagcgtctggaaggcatgccgcgcggtccccggtcctccttgtatgtgtgcagggtggccctggcgggggtctcctggctggaggaccccccatgcattacccctggaacctgcccctttgagcaccccccaccccacaacacacacgcacacacacaaacgcacgcacacgcacatactgcacacacattgcacacacgcagacacactgcacacacacacacacacacacacacacacacacacacacacacgctgcacagaggaaagtgccgtgcctgggtgggttggggcgggctccagaggaaggagccgcttgactcagagctacaggaagagccggggcaggcggggtgagaaccaccaactgcccgtcctcccgcccgcctagggaaggggtgggtgcctgggtggggtttagggttaggagaggatgtgactgcaaggccaggaagctacagggaaagttctgatcaaaatacacaaagacacaagccaggtccccaccgcgcttggcgatgcatccatagcagccttggtgctgtggacactccctggggcccagcgaaggggagagtttgctcccaaaggcgcaccaatgaccaacatttgccccccggaggaaagaactggaaccaggtgactgccttccccgctgctctgagtgagcctgtgtcagggcctggctgagaggaggcccacggcgcccaagacccatatgcatgtgtgtgcatgtgtgtgtgagacagagcgaggggcagcaggaggctgtgtcgcatcagcggccaagggtgggtgtcaggtgcagtgtgtgtgctgtggggtgcctgtggtcctaggctctgtgacaagcgttgcaatgggtgttgtatatactcaacagttgtgtgaggggtctgcagcctaagctgtgtgcagtggtaatgggaggtgtgtgtggtaggaagtgtgctgtgtaggaggtgcaagtgtgcacacgggctgagactgaagctctgtgcaggtgcacatgggccagagggctgtgtgtatgtgatgtgtgcaggggaggaggggcagaggagagggtgcaggggaagttagggaggggagggggtacaaggaaaggtgtgcaggggagagggtgcagggaaaggtggggaggggagagggtgcaggggaaggtaggcagaggagagggtgcaggggagagggtgcaggggaaggtgtgcagggaaaggtggggaggggagagggtgcaggggaaggtaggcagaggagagggtgcaggggaaggtgtgcaggggagagggtgcagggaaaggtggggaggggagagggtgcaggggaaggtaggcagaggagagggtgcaggggaaggtgtgcagggaaaggtggggagggagagggtgcaggggaaggtaggcagaggagagagtgcaggggaaggtgtgcaggggagagggtgcagggaaaggtggggaggggagagggtgcaggggaaggtaggcagacgagagtacagggaaaggtagggaggagagaaggtgcaggaggaggcaggcagaagagagggtgcaggggaaggtggggaggggagagggtgcagggggaggcaggcagaggagagggttcaggggagagggtgcaggggaaggtgggcaggggaaggtggggagtggagagcgtgcagggggaggcaggcagaggagagggtgcaggggaaggtgcgtaggggagagggagcaggggagagggtgcgggaagagggtgcaggggagggtttgcagggagagggtgcaggggagagggtgcaaggagaggcaggcagcggagagggtgcagaggagggtttgcaggggagggcacctgctttcttgctgtgctcgtatcctggcagtctgcccttgacttccagaaggctctgaggctgcttttggagggaggactttgaggtctgagcttggggcggtcacggaagcactgcaggagatgccaggggttctgctgggctggcggtgtgacctcccgggcttgctgtgaggggttggtttcctgggaagtgtgtgctttaaggaccctcagtgggtggttcccctgggtcaaggactttccttggagtgtcctccaccgcaaaggacttcttcaaggaccccctggccatcccccatgggtgtgtgcctcatgctgtatcggttcccgaggaaactgccaaacagtcaaacctggggcctctggctgtgcttcacccatggagagggaataggtggcaggctaagaggactgtccctgccactgcctctggggccttagcggggaggaatcctgagggagctggggtgcagaaacttaggcttgatccccacatccccacttccactgtgtccctgcagcagggaggggagtagacagtcagtgcctgttggataaacagggtgaccctgtggcatccagtgaggagaggcccctggggccctgggctgccaaggaagaggctctgggcttctccctgcagccacctcactgaggagctttgggagacttgaggtgtgtgtggctgctgctacgggctgggaaaggacatgggacccgagacctccatccccaccgggcgctgttcaccctccggcctcacaaccgcagggcgaggctaagctgagggttcccgaggtgtttcccgaggtgtttcgaggtgtctgtgctcacgtgcactcctgactgtaaccagacgtgggccagagctgggcaccccccctcgactgcatccagacatggttagagctgggcaccccccccccccgactgtatccagacatggtcagagctgagcacccctccccgactgtatccagacatgttcagagctgggcacccccccccgactgtatccagacatgttcagagctgggcacccccccccgactgtatccagacatggtcagagctgggcacccccccccgactgtatccagacatggtcagagctgggcaccccccgactgcatccagacatggtcagagctgagcacccccccccgcccgactgtatccagacatggtcagagctgggcaccccccgactgcatccagacatggtcagagctgggcacccccctccccgactgcattcagacatggtcagagctgggcacccccgccgactgcatccagacatggtcagagttgggcaccccccccccgactgtatccagacatggtcagagctgggcaccccccgactgcatccagacatggtcagagctgggcacccctccccgactgtatccagacatggtcagagctgggcacccccccccgactgtatccagacatggtcagagctgggcacctccccccgactgtatccagacatggtcagagctgggcacctcccccgactgcatccagacatggtcagagctgggcaccccccccgactgcatccagacatggtcagagctgggcaccccccccccccactgtatccagacatggtcagagctgggcacccccctccccgactgcatccagacatggtcagagctgagcaccccccccccccgactgtatccagacatggtcagagctgggcacccccctccccgactgtatccagacatggtcagagctgagccccccccccgcccgactgtatccagacatggtcagagctgggcaccccccgactgcatccagacatggtcagagctgagcacccctccccgactgcatccagacatggtcagagctgggcaccccccccccccaccgactgtatccagacatggtcagagctgggcaacccccaccgactgtatccagacatggtcagagctgggcaccccccgactgcatccagacatggtcagagctgggcaccccccgccgactgtatccagacatggtcagagctgggcacccccctccccgactgcatccagacatggtcagagctgggcacccccctccccgactgcatccagacatggtcagagctgggcacccctccccgactgtatccagacatggtcagagctgggcacccccctccccgactgtatccagacatggtcagagctgggcacccccgccgactgtatccagacatggtcagagctgggcaccccccgactgcatccagacatggtcagagctgggcacccctccccgactgtatccagacatggtcagagctgggcaccccccccccccgactgtatccagacatggtcagagctgagcacccctccccgactgtatccagacatgttcagagctgggcacccccccccccgactgtatccagacatggtcagagctgggcacccccctccccgactgcatccagacatggtcagagctgagcaccccccccgcccgactgcatccagacatggtcagagctgggcaccccccgactgcatccagacatggtcagagctgggcacccccctccccgactgcattcagacatggtcagagctgggcacccccctccccgactgcatccagacatggtcagagctgggcacccccgccgactgtatccagacatggtcagagctgggcacccccctccccgactgtatccagacatggtcagagctgggcacccccgccgactgtatccagacatggtcagagctgggcacccccctccccgactgcatccagacatgttcagagctgggcacccccccccgactgtatccagacatggtcagagctgggcaccccccgactgcatccagacatggtcagagctgggcaaccccctccctgactgcatccagacatggtcagagctgggcaccccccccggctgtatccagacatggtcagagctgggcaccccccccccccgactgcatccagacatggtcagagctaagcaaagccccccgccgactgtatccagacatggtcagagctgggcacccccaccccaactgcatccagacatggtcagagctgagcaccccccaccgactgtatccagacatggtcagagctgggcatctcccatggtgtaggttacatcactcacacccctgccccaaggccaggctgtgtctctggcactgcagcaccccctgcagtggcagctctgttgaaggggacagccaggagtgaggccaactgccatgtcgggagacagggtcccacctagtgttcgtccactgcaccctggggccgtcatggtggccccagggccggtggaggtgatcctggacttgatggcccctccccgtggtcctgggctgcgtgaagtggtgcccattctggccacgtgtgaggggctcaaagagacaccctgctggcctccgagaactctgccagcatccatgcggctgctcagggtcgcatctggtcagggccagtgctgtctgtggccggcagttactggttaactcatcctgttcctgtttaacttgttccctggggatggcggcagcctctgacctgtccaggtgccctgtccagctgactgcaaggacagagaggagtcctgcccagctcttggatcagtctgctggccgaggagcccggtggagccaggggtgaccctggagcccagcctgccccgaggaggccccggctcagagccatgccaggtaggcaggtcagagagggatgggcttgaattccccactcccacctcctgcccctcaggctggctccacattgtgcatcctgctcttatcccaggcactctgcctggccacatgccgggggtacaaaggcccctgctcacccctcccactgggcccttggccctgaaaccagggcgagtggtgaggatgagccctgcaccctctcctgccccagaccaggctcatgagggtcagtaaagcccaggaatgctaggagtgggcactgctggggcccacagcagggtgtggccgatgtgagctggcaggagaccataccctactgagaagatggtggtttgacctcccgctagggctcatcaccctgatgtaaagatgaacaagttcaggcctcaggtggtggggagggcttgcctgtggccaggagcagagggccccaagacccccaaggcaggaatgaggccaactgctccaggctcccagctgtgcccatccaggtggaaggtgctggcacactgggcatctgggtccccaaacccactggtgcccacactctctgcagattccccagcagaggcaggccaggctgaggggtgcagtgcccggcccctcctatgagacaggcatcatggtgtcaccaggggtgggcaacaggtgcatctgggaaatggggggctggactcacatcctgggtggacaagcagccagatggggcttgagcgtgggcctggggcagctcaactgtggccactgctctctgtcccctcagcacagggtgggcggaacacccaaagcctggccactactggggaaagacgtgccaagtgctaagcctgtccccatgggactcgtggacagacatggtgtgactgccaagccacacagaggccttatttcttcctgcaccacggaccactgtggaggtggtggggccaggcaccctggcacagctgacccactgtgtcctctctcttcaggtgtctgtgatagggcccctgacttcctctccccgtctgaagaccaggtgctgaggcctgccttgggcagctcagtggctctgaactgcacggcttgggtagtctctgggccccactgctccctgccttcagtccagtggctgaaagacgggcttccattgggaattgggggccactacagcctccacgagtactcctggtaagagacccgggtatccagggtcagagtgacctctcagacatgccaagggcagtggtctccctgacctatgcctgggtctgtaaccacctggccagacatgtcacgagcagagtgcctctgtggacccagacggagggtcagtaatgtcagggacagacccttgggtctgcatggcccctgtaggcacacacctcgtaactgcccagggctacgggtgtcagcaaagtctagggtctgaatgaacaccgaccagctggccaagtctgtgatcaaaggacctccaggccccagacccaggactgggacggctgttctgaaacaaatctgcatcccctccaggttcaggtcacttctcttggcttaaggcccaagaaccacccaggaggcccaattctgcagcctccctgggtgaacccagacaggtggggttcgggggtgtccactggtatccccagtcgaccctgaccctggcttggtatccccagggtcaaggccaacctgtcagaggtgcttgtgtccagtgtcctgggggtcaacgtgaccagcactgaagtctatggggccttcacctgctccatccagaacatcagcttctcctccttcactcttcagagagctggtgatgggggttccccaaggtggagggtagaaggggacctagacctagtgaggcccagggatcttgaggcttgggggctgctggaggggcagcggctcaggcaacccatccgcaggccctacaagccacgtggctgcggtgctggcctccctcctggtcctgctggccctgctgctggccgccctgctctatgtcaagtgccgtctcaacgtgctgctctggtaccaggacgcgtatggggaggtggagataaacggtgcgtggggcccgcgtgggcgcgaggaggggtcgccacggcctccctgagagtgcgctgctgagctcggctttggaggcgtgcggcggggaggggttagcccccgggtgctctgtgcggcccggctggggttaaagtccggggcgggtctgcccctgtgcacgtgggagatggttaggggtgttggggaccccgagggctggtgtgaggcctcgggagccatcggggtgactggccgccgtccgcagacgggaagctctacgacgcctacgtctcctacagcgactgccccgaggaccgcaagttcgtgaacttcatcctaagccgcagctggagcggcgtcggggctacaagctcttcctggacgaccgcgacctcctgccgcgcgctggtatcccgggccccaccccgtgccccgcccacccggagggcccgccccgccccgccccatgctccgtcccacccggggccccacccccaccatcgagctccgcccccatccccgcccacccgaggccccgcctcaaaaacccgcccaccccgcaggccccgcccctcccttagagctctgcgtccggcaccgcccctgagcctccggccccgccctcccccgcccccgcccctgcgccgccgacgcccgccctcccgcagagccctccgccgacctcttggtgaacctgagccgctgccgacgcctcatcgtggtgctttcggacgccttcctgagccgggcctggtgcagccacagcttccggtgggtcccgcgcggggttgggtgggccccagcgtagcacccacccccctgacggtcccgccccgcagggagggcctgtgccggctgctggagctcacccgcagacccatcttcatcaccttcgagggccagaggcgcgaccccgcgcacccggcgctccgcctgctgcgccagcaccgccacctggtgaccttgctgctctggaggcccggctccgtggtgcggagcaggcgcgggagggtccggggctagcggcgggttagagatgggcggtgcccgggctccaggctgggacccctccgtggggagctctgcggcaccacgctttgtgaatgggccctggggggaggttccgctgcctggggccccgatgcggggagccgcccttgaggcccccggagccacggaatagctgtcgcagggcgtggaacccgtgggcagccgcaggtgtgctcttgggggccaggacgccaggggcttccgaggtgttcacacctgcaaaccgccccgacctggcccccagactccttcctccgatttttggaaagaagtgcagctggcgctgccgcggaaggtgcagtacaggcctgtggaaggagacccccagacgcagctgcaggacgacaaggaccccatgctgattcttcgaggccgagtccctgagggccgggccctggactcagaggtggacccggaccctgagggcgacctgggtatgcccgcccagccccactccccaactggagaagctcagcacagggcggagtgggggcaggcacagggcacagggcctggaggggctccaggtgttgaggactcttcccggcaccgggagcccctgcacggcctctgccctggaggtgctcggccctcggtctgcctgggaacttcctgggcctcacaggccatcacagcagggggtgagcaggggcagcccctggcagtgggtctgggccaaggctgtgggtggccacctcaggcgtctcggtctccccaccccaggtgtccgggggcctgtctttggagagccatcagctccaccgcacaccagtggggtctcgctgggagagagccggagcagcgaagtggacgtctcggatctcggctcgcgaaactacagtgcccgcacagacttctactgcctggtgtccaaggatgatatgtagctcccaccccagagtgcaggatcatagggacagcgggggccagggcagcggcgtcgctcctctgctcaacaggaccacaacccctgccagcagccctgggaccctgccagcagccctgggaaaaggctgtggcctcagggcgcctcccagtgccagaaaataaagtccttttggattctg

SEQ ID NO: 3 - DNA, 1230 bp, Homo sapien
  wild type SIGIRR mRNA
augccaggugucugugauagggccccugacuuccucuccccgucugaagaccaggugcugaggccugccuugggcagcucaguggcucugaacugcacggcuuggguagucucugggccccacugcucccugccuucaguccaguggcugaaagacgggcuuccauugggaauugggggccacuacagccuccacgaguacuccugggucaaggccaaccugucagaggugcuuguguccaguguccugggggucaacgugaccagcacugaagucuauggggccuucaccugcuccauccagaacaucagcuucuccuccuucacucuucagagagcuggcccuacaagccacguggcugcggugcuggccucccuccugguccugcuggcccugcugcuggccgcccugcucuaugucaagugccgucucaacgugcugcucugguaccaggacgcguauggggagguggagauaaacgacgggaagcucuacgacgccuacgucuccuacagcgacugccccgaggaccgcaaguucgugaacuucauccuaaagccgcagcuggagcggcgucggggcuacaagcucuuccuggacgaccgcgaccuccugccgcgcgcugagcccuccgccgaccucuuggugaaccugagccgcugccgacgccucaucguggugcuuucggacgccuuccugagccgggccuggugcagccacagcuuccgggagggccugugccggcugcuggagcucacccgcagacccaucuucaucaccuucgagggccagaggcgcgaccccgcgcacccggcgcuccgccugcugcgccagcaccgccaccuggugaccuugcugcucuggaggcccggcuccgugacuccuuccuccgauuuuuggaaagaagugcagcuggcgcugccgcggaaggugcaguacaggccuguggaaggagacccccagacgcagcugcaggacgacaaggaccccaugcugauucuucgaggccgagucccugagggccgggcccuggacucagagguggacccggacccugagggcgaccuggguguccgggggccugucuuuggagagccaucagcuccaccgcacaccaguggggucucgcugggagagagccggagcagcgaaguggacgucucggaucucggcucgcgaaacuacagugcccgcacagacuucuacugccugguguccaaggaugauaug

SEQ ID NO: 4 - DNA, 645 bp, Homo sapien
  variant (c.557delA) SIGIRR mRNA
augccaggugucugugauagggccccugacuuccucuccccgucugaagaccaggugcugaggccugccuugggcagcucaguggcucugaacugcacggcuuggguagucucugggccccacugcucccugccuucaguccaguggcugaaagacgggcuuccauugggaauugggggccacuacagccuccacgaguacuccugggucaaggccaaccugucagaggugcuuguguccaguguccugggggucaacgugaccagcacugaagucuauggggccuucaccugcuccauccagaacaucagcuucuccuccuucacucuucagagagcuggcccuacaagccacguggcugcggugcuggccucccuccugguccugcuggcccugcugcuggccgcccugcucuaugucaagugccgucucaacgugcugcucugguaccaggacgcguauggggagguggagauaaacgacgggaagcucuacgacgccuacgucuccuacagcgacugccccgaggaccgcaaguucgugaacuucauccuaagccgcagcuggagcggcgucggggcuacaagcucuuccuggacgaccgcgaccuccugccgcgcgcugagcccuccgccgaccucuugg

SEQ ID NO: 5 - DNA, 1233 bp, Artificial Sequence
  wild type SIGIRR cDNA
atgccaggtgtctgtgatagggcccctgacttcctctccccgtctgaagaccaggtgctgaggcctgccttgggcagctcagtggctctgaactgcacggcttgggtagtctctgggccccactgctccctgccttcagtccagtggctgaaagacgggcttccattgggaattgggggccactacagcctccacgagtactcctgggtcaaggccaacctgtcagaggtgcttgtgtccagtgtcctgggggtcaacgtgaccagcactgaagtctatggggccttcacctgctccatccagaacatcagcttctcctccttcactcttcagagagctggccctacaagccacgtggctgcggtgctggcctccctcctggtcctgctggccctgctgctggccgccctgctctatgtcaagtgccgtctcaacgtgctgctctggtaccaggacgcgtatggggaggtggagataaacgacgggaagctctacgacgcctacgtctcctacagcgactgccccgaggaccgcaagttcgtgaacttcatcctaaagccgcagctggagcggcgtcggggctacaagctcttcctggacgaccgcgacctcctgccgcgcgctgagccctccgccgacctcttggtgaacctgagccgctgccgacgcctcatcgtggtgctttcggacgccttcctgagccgggcctggtgcagccacagcttccgggagggcctgtgccggctgctggagctcacccgcagacccatcttcatcaccttcgagggccagaggcgcgaccccgcgcacccggcgctccgcctgctgcgccagcaccgccacctggtgaccttgctgctctggaggcccggctccgtgactccttcctccgatttttggaaagaagtgcagctggcgctgccgcggaaggtgcagtacaggcctgtggaaggagacccccagacgcagctgcaggacgacaaggaccccatgctgattcttcgaggccgagtccctgagggccgggccctggactcagaggtggacccggaccctgagggcgacctgggtgtccgggggcctgtctttggagagccatcagctccaccgcacaccagtggggtctcgctgggagagagccggagcagcgaagtggacgtctcggatctcggctcgcgaaactacagtgcccgcacagacttctactgcctggtgtccaaggatgatatgtag

SEQ ID NO: 6 - DNA, 648 bp, Artificial Sequence
  variant (c.557delA) SIGIRR cDNA
atgccaggtgtctgtgatagggcccctgacttcctctccccgtctgaagaccaggtgctgaggcctgccttgggcagctcagtggctctgaactgcacggcttgggtagtctctgggccccactgctccctgccttcagtccagtggctgaaagacgggcttccattgggaattgggggccactacagcctccacgagtactcctgggtcaaggccaacctgtcagaggtgcttgtgtccagtgtcctgggggtcaacgtgaccagcactgaagtctatggggccttcacctgctccatccagaacatcagcttctcctccttcactcttcagagagctggccctacaagccacgtggctgcggtgctggcctccctcctggtcctgctggccctgctgctggccgccctgctctatgtcaagtgccgtctcaacgtgctgctctggtaccaggacgcgtatggggaggtggagataaacgacgggaagctctacgacgcctacgtctcctacagcgactgccccgaggaccgcaagttcgtgaacttcatcctaagccgcagctggagcggcgtcggggctacaagctcttcctggacgaccgcgacctcctgccgcgcgctgagccctccgccgacctcttggtga

SEQ ID NO: 7 - protein, 410 aa, Homo sapien
  wild type SIGIRR protein
MPGVCDRAPDFLSPSEDQVLRPALGSSVALNCTAWVVSGPHCSLPSVQWLKDGLPLGIGGHYSLHEYSWVKANLSEVLVSSVLGVNVTSTEVYGAFTCSIQNISFSSFTLQRAGPTSHVAAVLASLLVLLALLLAALLYVKCRLNVLLWYQDAYGEVEINDGKLYDAYVSYSDCPEDRKFVNFILKPQLERRRGYKLFLDDRDLLPRAEPSADLLVNLSRCRRLIVVLSDAFLSRAWCSHSFREGLCRLLELTRRPIFITFEGQRRDPAHPALRLLRQHRHLVTLLLWRPGSVTPSSDFWKEVQLALPRKVQYRPVEGDPQTQLQDDKDPMLILRGRVPEGRALDSEVDPDPEGDLGVRGPVFGEPSAPPHTSGVSLGESRSSEVDVSDLGSRNYSARTDFYCLVSKDDM

SEQ ID NO: 8 - protein, 504 aa, Homo sapien
  wild type SIGIRR isoform protein
MPGVCDRAPDFLSPSEDQVLRPALGSSVALNCTAWVVSGPHCSLPSVQWLKDGLPLGIGGHYSLHEYSWVKANLSEVLVSSVLGVNVTSTEVYGAFTCSIQNISFSSFTLQRAGPTSHVAAVLASLLVLLALLLAALLYVKCRLNVLLWYQDAYGEVEINDGKLYDAYVSYSDCPEDRKFVNFILKPQLERRRGYKLFLDDRDLLPRAEPSADLLVNLSRCRRLIVVLSDAFLSRAWCSHSFREGLCRLLELTRRPIFITFEGQRRDPAHPALRLLRQHRHLVTLLLWRPGSVTPSSDFWKEVQLALPRKVQYRPVEGDPQTQLQDDKDPMLILRGRVPEGRALDSEVDPDPEGDLGMPAQPHSPTGEAQHRAEWGQAQGTGPGGALGVEDSSRHREPLHGLCPGGARPSVCLGTSWASQAITAGGEQGQPLAVGLGQGCGWPPQASRSPHPRCPGACFWRAISSTAHQWGLAGREPEQRSGRLGSRLAKLQCPHRLLLPGVQG

SEQ ID NO: 9 - protein, 215 aa, Homo sapien
  Variant SIGIRR (c.557delA)
MPGVCDRAPDFLSPSEDQVLRPALGSSVALNCTAWVVSGPHCSLPSVQWLKDGLPLGIGGHYSLHEYSWVKANLSEVLVSSVLGVNVTSTEVYGAFTCSIQNISFSSFTLQRAGPTSHVAAVLASLLVLLALLLAALLYVKCRLNVLLWYQDAYGEVEINDGKLYDAYVSYSDCPEDRKFVNFILSRSWSGVGATSSSWTTATSCRALSPPPTSW

SEQ ID NO: 10 - protein, 30 aa, Homo sapien
  Wild type SIGIRR amio acids 186 to 215
KPQLERRRGYKLFLDDRDLLPRAEPSADLL

SEQ ID NO: 11 - protein, 30 aa, Homo sapien
  Variant SIGIRR amio acids 186 to 215
SRSWSGVGATSSSWTTATSCRALSPPPTSW

SEQ ID NO: 12 - DNA, 20 bp, Artificial Sequence
  forward PCR primer for SIGIRR
tcagtggctctgaactgcac

SEQ ID NO: 13 - DNA, 20 bp, Artificial Sequence
  reverse PCR primer for SIGIRR
ggtcctgttgagcagaggag

SEQ ID NO: 14 - protein, 910 aa, Artificial Sequence [sequence omitted]

SEQ ID NO: 15 - protein, 116 aa, Artificial Sequence
  heavy chain variable region of antibody directed to IL-6R
EVQLVESGGGLVQPGRSLRLSCAASRFTFDDYAMHWVRQAPGKGLEWVSGISWNSGRIGYADSVKGRFTISRDNAENSLFLQMNGLRAEDTALYYCAKGRDSFDIWGQGTMVTVSS

SEQ ID NO: 16 - protein, 107 aa, Artificial Sequence
  light chain variable region of antibody directed to IL-6R
DIQMTQSPSSVSASVGDRVTITCRASQGISSWLAWYQQKPGKAPKLLIYGASSLESGVPSRFSGSGSGTDFTLTISSLQPEDFASYYCQQANSFPYTFGQGTKLEIK